European Patent Application EP 4 582 440 A2, published July 9, 2025. Title: IL-10-CONTAINING VACCINES AND USES THEREOF. Applicant: The Regents of the University of California. Application EP. The sequence listing filed with the application follows.

SEQUENCE LISTING (14 sequences)

SEQ ID NO: 1 - DNA, 4148 bp, synthetic construct
  misc_feature 1..4148: note = Description of Artificial Sequence: Synthetic polynucleotide
  source 1..4148: mol_type = other DNA
cgtgaggctccggtgcccgtcagtgggcagagcgcacatcgcccacagtccccgagaagttggggggagggatcggcaattgaaccggtgcctagagaaggtggcgcggggtaaactgggaaagtgatgtcgtgtactggctccgcctttttcccgagggtgggggagaaccgtatataagtgcagtagtcgccgtgaacgttctttttcgcaacgggtttgccgccagaacacaggtaagtgccgtgtgtggttcccgcgggcctggcctctttacgggttatggcccttgcgtgccttgaattacttccacctggctgcagtacgtgattcttgatcccgagcttcgggttggaagtgggtgggagagttcgaggccttgcgcttaaggagccccttcgcctcgtgcttgagttgaggcctggcctgggcgctggggccgccgcgtgcgaatctggtggcaccttcgcgcctgtctcgctgctttcgataagtctctagccatttaaaatttttgatgacctgctgcgacgctttttttctggcaagatagtcttgtaaatgcgggccaagatctgcacactggtatttcggtttttggggccgcgggcggcgacggggcccgtgcgtcccagcgcacatgttcggcgaggcggggcctgcgagcgcggccaccgagaatcggacgggggtagtctcaagctggccggcctgctctggtgcctggcctcgcgccgccgtgtatcgccccgccctgggcggcaaggctggcccggtcggcaccagttgcgtgagcggaaagatggccgcttcccggccctgctgcagggagctcaaaatggaggacgcggcgctcgggagagcgggcgggtgagtcacccacacaaaggaaaagggcctttccgtcctcagccgtcgcttcatgtgactccacggagtaccgggcgccgtccaggcacctcgattagttctcgagcttttggagtacgtcgtctttaggttggggggaggggttttatgcgatggagtttccccacactgagtgggtggagactgaagttaggccagcttggcacttgatgtaattctccttggaatttgccctttttgagtttggatcttggttcattctcaagcctcagacagtggttcaaagtttttttcttccatttcaggtgtcgtgaggaattagctggcgcgccttcccgccaccatgggcgtgagaaactccgtcttgtcagggaagaaagcagatgaattagaaaaaattaggctacgacccaacggaaagaaaaagtacatgttgaagcatgtagtatgggcagcaaatgaattagatagatttggattagcagaaagcctgttggagaacaaagaaggatgtcaaaaaatactttcggtcttagctccattagtgccaacaggctcagaaaatttaaaaagcctttataatactgtctgcgtcatctggtgcattcacgcagaagagaaagtgaaacacactgaggaagcaaaacagatagtgcagagacacctagtggtggaaacaggaaccaccgaaaccatgccgaagacctctcgaccaacagcaccatctagcggcagaggaggaaactacccagtacagcagatcggtggcaactacgtccacctgccactgtccccgagaaccctgaacgcttgggtcaagctgatcgaggagaagaagttcggagcagaagtagtgccaggattccaggcactgtcagaaggttgcaccccctacgacatcaaccagatgctgaactgcgttggagaccatcaggcggctatgcagatcatccgtgacatcatcaacgaggaggctgcagattgggacttgcagcacccacaaccagctccacaacaaggacaacttagggagccgtcaggatcagacatcgcaggaaccacctcctcagttgacgaacagatccagtggatgtaccgtcagcagaacccgatcccagtaggcaacatctaccgtcgatggatccagctgggtctgcagaaatgcgtccgtatgtacaacccgaccaacattctagatgtaaaacaagggccaaaagagccatttcagagctatgtagacaggttctacaaaagtttaagagcagaacagacagatgcagcagtaaagaattggatgactcaaacactgctgattcaaaatgctaacccagattgcaagctagtgctgaaggggctgggtgtgaatcccaccctagaagaaatgctgacggcttgtcaaggagtaggggggccgggacagaaggctagattaatggcagaagccctgaaagaggccctcgcaccagtgccaatcccttttgcagcagcccaacagaggggaccaagaaagccaattaagtgttggaattgtgggaaagagggacactctgcaaggcaatgcagagccccaagaagacagggatgctggaaatgtggaaaaatggaccatgttatggccaaatgcccagacagacaggcgggttttttaggccttggtccatggggaaagaagccccgcaatttccccatggctcaagtgcatcaggggctgatgccaactgctcccccagaggacccagctgtggatctgctaaagaactacatgcagttgggcaagcagcagagagaaaagcagagagaaagcagagagaagccttacaaggaggtgacagaggatttgctgcacctcaattctctctttggaggagaccaggactacaaagacgatgacgacaagtagtagcctgcaggcccctctccctcccccccccctaacgttactggccgaagccgcttggaataaggccggtgtgcgtttgtctatatgttattttccaccatattgccgtcttttggcaatgtgagggcccggaaacctggccctgtcttcttgacgagcattcctaggggtctttcccctctcgccaaaggaatgcaaggtctgttgaatgtcgtgaaggaagcagttcctctggaagcttcttgaagacaaacaacgtctgtagcgaccctttgcaggcagcggaaccccccacctggcgacaggtgcctctgcggccaaaagccacgtgtataagatacacctgcaaaggcggcacaaccccagtgccacgttgtgagttggatagttgtggaaagagtcaaatggctctcctcaagcgtattcaacaaggggctgaaggatgcccagaaggtaccccattgtatgggatctgatctggggcctcggtgcacatgctttacatgtgtttagtcgaggttaaaaaaacgtctaggccccccgaaccacggggacgtggttttcctttgaaaaacacgatgataaagccaccatgcacagctcagcactgctctgttgcctagtcctcctgactggggtgagggccagcccaggccagggcacccagtctgagaacagctgcacccgcttcccaggcaacctgcctcacatgcttcgagacctccgagatgccttcagcagagtgaagactttctttcaaatgaaggatcagctggacaacatattgttaaaggagtccttgctggaggactttaagggttacctgggttgccaagccttgtctgagatgatccagttttacctggaggaggtgatgccccaagctgagaaccacgacccagacatcaaggagcatgtgaactccctgggggagaatctgaagaccctcaggctgaggctgcggcgctgtcatcgatttcttccctgtgaaaacaagagcaaggccgtggagcaggtgaagaatgcctttagtaagctccaagagaaaggcgtctacaaagccatgagtgagtttgacatcttcatcaactacatagaagcctacatgacaatgaagatacaaaactgagacctgcaggacgccacagctctgatcataatcagccataccacatttgtagaggttttacttgctttaaaaaacctcccacacctccccctgaacctgaaacataaaatgaatgcaattgttgttgttaacttgtttattgcagcttataatggttacaaataaagcaatagcatcacaaatttcacaaataaagcatttttttcactgcattctagttgtggtttgtccaaactcatcaatgtatct

SEQ ID NO: 2 - protein, 509 aa, synthetic construct
  REGION 1..509: note = Description of Artificial Sequence: Synthetic polypeptide
MGVRNSVLSGKKADELEKIRLRPNGKKKYMLKHVVWAANELDRFGLAESLLENKEGCQKILSVLAPLVPTGSENLKSLYNTVCVIWCIHAEEKVKHTEEAKQIVQRHLVVETGTTETMPKTSRPTAPSSGRGGNYPVQQIGGNYVHLPLSPRTLNAWVKLIEEKKFGAEVVPGFQALSEGCTPYDINQMLNCVGDHQAAMQIIRDIINEEAADWDLQHPQPAPQQGQLREPSGSDIAGTTSSVDEQIQWMYRQQNPIPVGNIYRRWIQLGLQKCVRMYNPTNILDVKQGPKEPFQSYVDRFYKSLRAEQTDAAVKNWMTQTLLIQNANPDCKLVLKGLGVNPTLEEMLTACQGVGGPGQKARLMAEALKEALAPVPIPFAAAQQRGPRKPIKCWNCGKEGHSARQCRAPRRQGCWKCGKMDHVMAKCPDRQAGFLGLGPWGKKPRNFPMAQVHQGLMPTAPPEDPAVDLLKNYMQLGKQQREKQRESREKPYKEVTEDLLHLNSLFGGD

SEQ ID NO: 3 - protein, 8 aa, synthetic construct
  REGION 1..8: note = Description of Artificial Sequence: Synthetic peptide
DYKDDDDK

SEQ ID NO: 4 - protein, 178 aa, Macaca mulatta
MHSSALLCCLVLLTGVRASPGQGTQSENSCTRFPGNLPHMLRDLRDAFSRVKTFFQMKDQLDNILLKESLLEDFKGYLGCQALSEMIQFYLEEVMPQAENHDPDIKEHVNSLGENLKTLRLRLRRCHRFLPCENKSKAVEQVKNAFSKLQEKGVYKAMSEFDIFINYIEAYMTMKIQN

SEQ ID NO: 5 - DNA, 1175 bp, Cercopithecine herpesvirus 8
  source 1..1175: mol_type = genomic DNA
atgcggaggaggaggaggtctttcggcatcatcgtcgccggcgctatcggaacactactcatgatggcggtggtcgtgctttcagcccatgaccatgaacacaaagaagtaccaccggcctgtgaccccgttcacggtaacttggcaggcatcttcaaggagttgcgggcgacctacgcttccattagagaaggtttggtatgttaggcaacgcagttctcggatgtcagtccggatcggaggagtcacagtctgtcatgtgatgatatattgcttaatttttgttttgcagcaaaagaaggacacggtgtactacacatcgctgttcaatgaccgcgtgctccatgaaatgctgagtcctatgggctgtcgcgtgaccaatgaactcatggaacattatttagatggtgttctgcctcgagcaagtcatttagactacgataatagcactctgaatggcttacatgtgtttgcttcatccatgcaggcgctgtatcagcacatgttaaagtgtgtaagtgtttcaggttcgataaccccgcgatatgacacgtaaatagcgatatcgtggcaccagacgtcagtcacagtcttccccggtcgagacgcatcttatatcgcgatatatcgcggattatcgcagtatgtagcgatatatcgtgtcaaagcactccgaacgacattctgatgacggctatcgccttatgtcgcggtatatcgcggaatatcgcagtatatcgcggttatgtcgcgacataaccgtcatgtcgcgactatcgccgcatatcgccactatcgcgacttggcaccgtgccaacgatagtcgaccttagggtggtcgtgtggtggtggggggctgcttgcggtttgcaaaccggagaggtagcacacgctgattgtcggtttggaagcgttgtttacacatgtctttgtcttggcagcccgcgttggcatgtactggcaaaacgccagcttggatgtacttcttggaggtggaacacaaggtcagttaaggttgccaggtaggttaaaacgcagaaaccattgttctaccggtttcctaaaacgccgttcaacgtgttttgcagctcaacccctggaggggcacggcaaaagccgcggccgaggctgaccttttgctgaactacttggaaacgttcctgctgcagttctga

SEQ ID NO: 6 - DNA, 1179 bp, Cercopithecine herpesvirus 8
  source 1..1179: mol_type = genomic DNA
atgcggaggaggaggaggtctttcggcatcatcgtcgccggcgctatcggaacactactcatgatggcggtggtcgtgctttcagcccatgaacacaaagaagtaccaccggcctgtgaccccgttcacggtaacttggcaggcatcttcaaggagttgcgggcgacctacgcttccattagagaaggtttggtatgttaggcaacgcagttctcggatgtcagtccggatcggaggagtcacagtctgtcatgtgatgatatattgcttcatttttgttttgcagcaaaagaaggacacggtgtactacacatcgctgttcaatgaccgcgtgctccatgagatgctgagtcctatgggctgtcgcgtgaccaacgaactcatggaacattatttagatggtgttctgcctcgagcaagtcatttagactacgataatagcactctgaatggcttacatgtgtttgcttcatccatgcaggcgctgtatcagcacatgttaaagtgtgtaagtgtttcaggttcgataaccccgcgatatgacacgtaaatagcgatatcgtggcaccagacgtcagtcacagtcttccccggtcgagacgcatcttatatcgcgatatatcgcggtttatcgcagtatgtcgcgatatatcgctccaaaacactccggatgactttctatcgccgaatatcacctcatatcgtcttatatcgcggtgtatcgcgggttatcgtcatatatcgcggttatgtcgcgacataaccgtcatgtcgcgactatcgccgcatatcgccactatcgcgacttggcacggtgccaacaatagttgcctctagggtggtcgtgtggtggtagggggctgcttacggtttgcaaaccggagaggtcgcacacgctgattgtcggtttggaagcgttgtttacacatgtctttgtcttggcagcccgcgttggcatgtactggcaaaacgccagcttggatgtacttcttggaggtggaacacaaggtcagttaaggttgccaggtaggttaaaacgcagaaaccattgttctaccggtttcctaaaacgccgttcaacgtgttttgcagctcaacccctggaggggcacggcaaaagccgcggccgaggctgaccttttgctgaactacttggaaacgttcctgctgcagttctga

SEQ ID NO: 7 - protein, 178 aa, Homo sapiens
MHSSALLCCLVLLTGVRASPGQGTQSENSCTHFPGNLPNMLRDLRDAFSRVKTFFQMKDQLDNLLLKESLLEDFKGYLGCQALSEMIQFYLEEVMPQAENQDPDIKAHVNSLGENLKTLRLRLRRCHRFLPCENKSKAVEQVKNAFNKLQEKGIYKAMSEFDIFINYIEAYMTMKIRN

SEQ ID NO: 8 - DNA, 3545 bp, synthetic construct
  misc_feature 1..3545: note = Description of Artificial Sequence: Synthetic polynucleotide
  source 1..3545: mol_type = other DNA
cgtgaggctccggtgcccgtcagtgggcagagcgcacatcgcccacagtccccgagaagttggggggagggatcggcaattgaaccggtgcctagagaaggtggcgcggggtaaactgggaaagtgatgtcgtgtactggctccgcctttttcccgagggtgggggagaaccgtatataagtgcagtagtcgccgtgaacgttctttttcgcaacgggtttgccgccagaacacaggtaagtgccgtgtgtggttcccgcgggcctggcctctttacgggttatggcccttgcgtgccttgaattacttccacctggctgcagtacgtgattcttgatcccgagcttcgggttggaagtgggtgggagagttcgaggccttgcgcttaaggagccccttcgcctcgtgcttgagttgaggcctggcctgggcgctggggccgccgcgtgcgaatctggtggcaccttcgcgcctgtctcgctgctttcgataagtctctagccatttaaaatttttgatgacctgctgcgacgctttttttctggcaagatagtcttgtaaatgcgggccaagatctgcacactggtatttcggtttttggggccgcgggcggcgacggggcccgtgcgtcccagcgcacatgttcggcgaggcggggcctgcgagcgcggccaccgagaatcggacgggggtagtctcaagctggccggcctgctctggtgcctgtcctcgcgccgccgtgtatcgccccgccctgggcggcaaggctggcccggtcggcaccagttgcgtgagcggaaagatggccgcttcccggccctgctgcagggagctcaaaatggaggacgcggcgctcgggagagcgggcgggtgagtcacccacacaaaggaaaagggcctttccgtcctcagccgtcgcttcatgtgactccacggagtaccgggcgccgtccaggcacctcgattagttctcgagcttttggagtacgtcgtctttaggttggggggaggggttttatgcgatggagtttccccacactgagtgggtggagactgaagttaggccagcttggcacttgatgtaattctccttggaatttgccctttttgagtttggatcttggttcattctcaagcctcagacagtggttcaaagtttttttcttccatttcaggtgtcgtgaggaattagctggcgcgccttcccgccaccatgtcttctgagcagaagagtcagcactgcaagcctgaggaaggcgttgaggcccaagaagaggccctgggcctggtgggtgcacaggctcctactactgaggagcaggaggctgctgtctcctcctcctctcctctggtccctggcaccctggaggaagtgcctgctgctgagtcagcaggtcctccccagagtcctcagggagcctctgccttacccactaccatcagcttcacttgctggaggcaacccaatgagggttccagcagccaagaagaggaggggccaagcacctcgcctgacgcagagtccttgttccgagaagcactcagtaacaaggtggatgagttggctcattttctgctccgcaagtatcgagccaaggagctggtcacaaaggcagaaatgctggagagagtcatcaaaaattacaagcgctgctttcctgtgatcttcggcaaagcctccgagtccctgaagatgatctttggcattgacgtgaaggaagtggaccccgccagcaacacctacacccttgtcacctgcctgggcctttcctatgatggcctgctgggtaataatcagatctttcccaagacaggccttctgataatcgtcctgggcacaattgcaatggagggcgacagcgcctctgaggaggaaatctgggaggagctgggtgtgatgggggtgtatgatgggagggagcacactgtctatggggagcccaggaaactgctcacccaagattgggtgcaggaaaactacctggagtaccggcaggtacccggcagtaatcctgcgcgctatgagttcctgtggggtccaagggctctggctgaaaccagctatgtgaaagtcctggagcatgtggtcagggtcaatgcaagagttcgcattgcctacccatccctgcgtgaagcagctttgttagaggaggaagagggagtctgatagcctgcaggcccctctccctcccccccccctaacgttactggccgaagccgcttggaataaggccggtgtgcgtttgtctatatgttattttccaccatattgccgtcttttggcaatgtgagggcccggaaacctggccctgtcttcttgacgagcattcctaggggtctttcccctctcgccaaaggaatgcaaggtctgttgaatgtcgtgaaggaagcagttcctctggaagcttcttgaagacaaacaacgtctgtagcgaccctttgcaggcagcggaaccccccacctggcgacaggtgcctctgcggccaaaagccacgtgtataagatacacctgcaaaggcggcacaaccccagtgccacgttgtgagttggatagttgtggaaagagtcaaatggctctcctcaagcgtattcaacaaggggctgaaggatgcccagaaggtaccccattgtatgggatctgatctggggcctcggtgcacatgctttacatgtgtttagtcgaggttaaaaaaacgtctaggccccccgaaccacggggacgtggttttcctttgaaaaacacgatgataaagccaccatgcacagctcagcactgctctgttgcctagtcctcctgactggggtgagggccagcccaggccagggcacccagtctgagaacagctgcacccgcttcccaggcaacctgcctcacatgcttcgagacctccgagatgccttcagcagagtgaagactttctttcaaatgaaggatcagctggacaacatattgttaaaggagtccttgctggaggactttaagggttacctgggttgccaagccttgtctgagatgatccagttttacctggaggaggtgatgccccaagctgagaaccacgacccagacatcaaggagcatgtgaactccctgggggagaatctgaagaccctcaggctgaggctgcggcgctgtcatcgatttcttccctgtgaaaacaagagcaaggccgtggagcaggtgaagaatgcctttagtaagctccaagagaaaggcgtctacaaagccatgagtgagtttgacatcttcatcaactacatagaagcctacatgacaatgaagatacaaaactgagacctgcaggacgccacagctctgatcataatcagccataccacatttgtagaggttttacttgctttaaaaaacctcccacacctccccctgaacctgaaacataaaatgaatgcaattgttgttgttaacttgtttattgcagcttataatggttacaaataaagcaatagcatcacaaatttcacaaataaagcatttttttcactgcattctagttgtggtttgtccaaactcatcaatgtatct

SEQ ID NO: 9 - DNA, 3701 bp, synthetic construct
  misc_feature 1..3701: note = Description of Artificial Sequence: Synthetic polynucleotide
  source 1..3701: mol_type = other DNA
cgtgaggctccggtgcccgtcagtgggcagagcgcacatcgcccacagtccccgagaagttggggggagggatcggcaattgaaccggtgcctagagaaggtggcgcggggtaaactgggaaagtgatgtcgtgtactggctccgcctttttcccgagggtgggggagaaccgtatataagtgcagtagtcgccgtgaacgttctttttcgcaacgggtttgccgccagaacacaggtaagtgccgtgtgtggttcccgcgggcctggcctctttacgggttatggcccttgcgtgccttgaattacttccacctggctgcagtacgtgattcttgatcccgagcttcgggttggaagtgggtgggagagttcgaggccttgcgcttaaggagccccttcgcctcgtgcttgagttgaggcctggcctgggcgctggggccgccgcgtgcgaatctggtggcaccttcgcgcctgtctcgctgctttcgataagtctctagccatttaaaatttttgatgacctgctgcgacgctttttttctggcaagatagtcttgtaaatgcgggccaagatctgcacactggtatttcggtttttggggccgcgggcggcgacggggcccgtgcgtcccagcgcacatgttcggcgaggcggggcctgcgagcgcggccaccgagaatcggacgggggtagtctcaagctggccggcctgctctggtgcctgtcctcgcgccgccgtgtatcgccccgccctgggcggcaaggctggcccggtcggcaccagttgcgtgagcggaaagatggccgcttcccggccctgctgcagggagctcaaaatggaggacgcggcgctcgggagagcgggcgggtgagtcacccacacaaaggaaaagggcctttccgtcctcagccgtcgcttcatgtgactccacggagtaccgggcgccgtccaggcacctcgattagttctcgagcttttggagtacgtcgtctttaggttggggggaggggttttatgcgatggagtttccccacactgagtgggtggagactgaagttaggccagcttggcacttgatgtaattctccttggaatttgccctttttgagtttggatcttggttcattctcaagcctcagacagtggttcaaagtttttttcttccatttcaggtgtcgtgaggaattagctggcgcgccttcccgccaccatgcctcgagctccaaagcgtcagcgctgcatgcctgaagaagatcttcaatcccaaagtgagacacagggcctcgagggtgcacaggctcccctggctgtggaggaggatgcttcatcatccacttccaccagctcctcttttccatcctcttttccctcctcctcctcttcctcctcctcctcctgctatcctctaataccaagcaccccagaggaggtttctgctgatgatgagacaccaaatcctccccagagtgctcagatagcctgctcctccccctcggtcgttgcttcccttccattagatcaatctgatgagggctccagcagccaaaaggaggagagtccaagcaccctacaggtcctgccagacagtgagtctttacccagaagtgagatagatgaaaaggtgactgatttggtgcagtttctgctcttcaagtatcaaatgaaggagccgatcacaaaggcagaaatactggagagtgtcataagaaattatgaagaccacttccctttgttgtttagtgaagcctccgagtgcatgctgctggtctttggcattgatgtaaaggaagtggatcccactggccactcctttgtccttgtcacctccctgggcctcacctatgatgggatgctgagtgatgtccagagcatgcccaagactggcattctcatacttatcctaagcatagtcttcatagagggctactgcacccctgaggaggtcatctgggaagcactgaatatgatggggctgtatgatgggatggagcacctcatttatggggagcccaggaagctgctcacccaagattgggtgcaggaaaactacctggagtaccggcaggtgcctggcagtgatcctgcacggtatgagtttctgtggggtccaagggctcatgctgaaattaggaagatgagtctcctgaaatttttggccaaggtaaatgggagtgatccaagatccttcccactgtggtatgaggaggctttgaaagatgaggaagagagagcccaggacagaattgccaccacagatgatactactgccatggccagtgcaagttctagcgctacaggtagcttctcctaccctgaataatagcctgcaggcccctctccctcccccccccctaacgttactggccgaagccgcttggaataaggccggtgtgcgtttgtctatatgttattttccaccatattgccgtcttttggcaatgtgagggcccggaaacctggccctgtcttcttgacgagcattcctaggggtctttcccctctcgccaaaggaatgcaaggtctgttgaatgtcgtgaaggaagcagttcctctggaagcttcttgaagacaaacaacgtctgtagcgaccctttgcaggcagcggaaccccccacctggcgacaggtgcctctgcggccaaaagccacgtgtataagatacacctgcaaaggcggcacaaccccagtgccacgttgtgagttggatagttgtggaaagagtcaaatggctctcctcaagcgtattcaacaaggggctgaaggatgcccagaaggtaccccattgtatgggatctgatctggggcctcggtgcacatgctttacatgtgtttagtcgaggttaaaaaaacgtctaggccccccgaaccacggggacgtggttttcctttgaaaaacacgatgataaagccaccatgcacagctcagcactgctctgttgcctagtcctcctgactggggtgagggccagcccaggccagggcacccagtctgagaacagctgcacccgcttcccaggcaacctgcctcacatgcttcgagacctccgagatgccttcagcagagtgaagactttctttcaaatgaaggatcagctggacaacatattgttaaaggagtccttgctggaggactttaagggttacctgggttgccaagccttgtctgagatgatccagttttacctggaggaggtgatgccccaagctgagaaccacgacccagacatcaaggagcatgtgaactccctgggggagaatctgaagaccctcaggctgaggctgcggcgctgtcatcgatttcttccctgtgaaaacaagagcaaggccgtggagcaggtgaagaatgcctttagtaagctccaagagaaaggcgtctacaaagccatgagtgagtttgacatcttcatcaactacatagaagcctacatgacaatgaagatacaaaactgagacctgcaggacgccacagctctgatcataatcagccataccacatttgtagaggttttacttgctttaaaaaacctcccacacctccccctgaacctgaaacataaaatgaatgcaattgttgttgttaacttgtttattgcagcttataatggttacaaataaagcaatagcatcacaaatttcacaaataaagcatttttttcactgcattctagttgtggtttgtccaaactcatcaatgtatct

SEQ ID NO: 10 - protein, 770 aa, Homo sapiens
MAQWNQLQQLDTRYLEQLHQLYSDSFPMELRQFLAPWIESQDWAYAASKESHATLVFHNLLGEIDQQYSRFLQESNVLYQHNLRRIKQFLQSRYLEKPMEIARIVARCLWEESRLLQTAATAAQQGGQANHPTAAVVTEKQQMLEQHLQDVRKRVQDLEQKMKVVENLQDDFDFNYKTLKSQGDMQDLNGNNQSVTRQKMQQLEQMLTALDQMRRSIVSELAGLLSAMEYVQKTLTDEELADWKRRQQIACIGGPPNICLDRLENWITSLAESQLQTRQQIKKLEELQQKVSYKGDPIVQHRPMLEERIVELFRNLMKSAFVVERQPCMPMHPDRPLVIKTGVQFTTKVRLLVKFPELNYQLKIKVCIDKDSGDVAALRGSRKFNILGTNTKVMNMEESNNGSLSAEFKHLTLREQRCGNGGRANCDASLIVTEELHLITFETEVYHQGLKIDLETHSLPVVVISNICQMPNAWASILWYNMLTNNPKNVNFFTKPPIGTWDQVAEVLSWQFSSTTKRGLSIEQLTTLAEKLLGPGVNYSGCQITWAKFCKENMAGKGFSFWVWLDNIIDLVKKYILALWNEGYIMGFISKERERAILSTKPPGTFLLRFSESSKEGGVTFTWVEKDISGKTQIQSVEPYTKQQLNNMSFAEIIMGYKIMDATNILVSPLVYLYPDIPKEEAFGKYCRPESQEHPEADPGSAAPYLKTKFICVTPTTCSNTIDLPMSPRTLDSLMQFGNNGEGAEPSAGGQFESLTFDMELTSECATSPM

SEQ ID NO: 11 - protein, 874 aa, Macaca mulatta
MTACPGQAGAGRGLAEGAVIQRFPELRRRRPGGGAGGSDVAAEGTSPNRILDRHPGSALSLPLGSDKPSGLREPRRPPPAHAQPRPLGLCWRNSRMAQWNQLQQLDTRYLEQLHQLYSDSFPMELRQFLAPWIESQDWAYAASKESHATLVFHNLLGEIDQQYSRFLQESNVLYQHNLRRIKQFLQSRYLEKPMEIARIVARCLWEESRLLQTAATAAQQGGQANHPTAAVVTEKQQMLEQHLQDVRKRVQDLEQKMKVVENLQDDFDFNYKTLKSQGGQGVSPSSADMQDLNGNNQSVTRQKMQQLEQMLTALDQMRRSIVSELAGLLSAMEYVQKTLTDEELADWKRRQQIACIGGPPNICLDRLENWITSLAESQLQTRQQIKKLEELQQKVSYKGDPIVQHRPMLEERIVELFRNLMKSAFVVERQPCMPMHPDRPLVIKTGVQFTTKVRLLVKFPELNYQLKIKVCIDKDSGDVAALRGSRKFNILGTNTKVMNMEESNNGSLSAEFKHLTLREQRCGNGGRANCDASLIVTEELHLITFETEVYHQGLKIDLETHSLPVVVISNICQMPNAWASILWYNMLTNNPKNVNFFTKPPIGTWDQVAEVLSWQFSSTTKRGLSIEQLTTLAEKLLGPGVNYSGCQITWAKFCKENMAGKGFSFWVWLDNIIDLVKKYILALWNEGYIMGFISKERERAILSTKPPGTFLLRFSESSKEGGVTFTWVEKDISGKTQIQSVEPYTKQQLNNMSFAEIIMGYKIMDATNILVSPLVYLYPDIPKEEAFGKYCRPESQEHPEADPGSAAPYLKTKFICVTPTTCSNTIDLPMSPRTLDSLMQFGNNGEGAEPSAGGQFESLTFDMELTSECATSPM

SEQ ID NO: 12 - protein, 770 aa, Homo sapiens
MAQWNQLQQLDTRYLEQLHQLYSDSFPMELRQFLAPWIESQDWAYAASKESHATLVFHNLLGEIDQQYSRFLQESNVLYQHNLRRIKQFLQSRYLEKPMEIARIVARCLWEESRLLQTAATAAQQGGQANHPTAAVVTEKQQMLEQHLQDVRKRVQDLEQKMKVVENLQDDFDFNYKTLKSQGDMQDLNGNNQSVTRQKMQQLEQMLTALDQMRRSIVSELAGLLSAMEYVQKTLTDEELADWKRRQQIACIGGPPNICLDRLENWITSLAESQLQTRQQIKKLEELQQKVSYKGDPIVQHRPMLEERIVELFRNLMKSAFVVERQPCMPMHPDRPLVIKTGVQFTTKVRLLVKFPELNYQLKIKVCIDKDSGDVAALRGSRKFNILGTNTKVMNMEESNNGSLSAEFKHLTLREQRCGNGGRANCDASLIVTEELHLITFETEVYHQGLKIDLETHSLPVVVISNICQMPNAWASILWYNMLTNNPKNVNFFTKPPIGTWDQVAEVLSWQFSSTTKRGLSIEQLTTLAEKLLGPGVNYSGCQITWAKFCKENMAGKGFSFWVWLDNIIDLVKKYILALWNEGYIMGFISKERERAILSTKPPGTFLLRFSESSKEGGVTFTWVEKDISGKTQIQSVEPYTKQQLNNMSFAEIIMGYKIMDCTCILVSPLVYLYPDIPKEEAFGKYCRPESQEHPEADPGSAAPYLKTKFICVTPTTCSNTIDLPMSPRTLDSLMQFGNNGEGAEPSAGGQFESLTFDMELTSECATSPM

SEQ ID NO: 13 - protein, 874 aa, Macaca mulatta
MTACPGQAGAGRGLAEGAVIQRFPELRRRRPGGGAGGSDVAAEGTSPNRILDRHPGSALSLPLGSDKPSGLREPRRPPPAHAQPRPLGLCWRNSRMAQWNQLQQLDTRYLEQLHQLYSDSFPMELRQFLAPWIESQDWAYAASKESHATLVFHNLLGEIDQQYSRFLQESNVLYQHNLRRIKQFLQSRYLEKPMEIARIVARCLWEESRLLQTAATAAQQGGQANHPTAAVVTEKQQMLEQHLQDVRKRVQDLEQKMKVVENLQDDFDFNYKTLKSQGGQGVSPSSADMQDLNGNNQSVTRQKMQQLEQMLTALDQMRRSIVSELAGLLSAMEYVQKTLTDEELADWKRRQQIACIGGPPNICLDRLENWITSLAESQLQTRQQIKKLEELQQKVSYKGDPIVQHRPMLEERIVELFRNLMKSAFVVERQPCMPMHPDRPLVIKTGVQFTTKVRLLVKFPELNYQLKIKVCIDKDSGDVAALRGSRKFNILGTNTKVMNMEESNNGSLSAEFKHLTLREQRCGNGGRANCDASLIVTEELHLITFETEVYHQGLKIDLETHSLPVVVISNICQMPNAWASILWYNMLTNNPKNVNFFTKPPIGTWDQVAEVLSWQFSSTTKRGLSIEQLTTLAEKLLGPGVNYSGCQITWAKFCKENMAGKGFSFWVWLDNIIDLVKKYILALWNEGYIMGFISKERERAILSTKPPGTFLLRFSESSKEGGVTFTWVEKDISGKTQIQSVEPYTKQQLNNMSFAEIIMGYKIMDCTCILVSPLVYLYPDIPKEEAFGKYCRPESQEHPEADPGSAAPYLKTKFICVTPTTCSNTIDLPMSPRTLDSLMQFGNNGEGAEPSAGGQFESLTFDMELTSECATSPM

SEQ ID NO: 14 - protein, 10 aa, synthetic construct
  REGION 1..10: note = Description of Artificial Sequence: Synthetic His tag
  REGION 1..10: note = MISC_FEATURE - This sequence may encompass 6-10 residues
HHHHHHHHHH